European Patent Specification EP 4 060 037 B1, published August 21, 2024. Title: Novel tautomerase pptA variant and a method for producing L-tryptophan using the same. Applicant: CJ CheilJedang Corporation. The sequence listing filed with the application follows.

SEQUENCE LISTING (10 sequences)

SEQ ID NO: 1 - protein, 77 aa, Artificial Sequence
  pptA
MPHIDIKCFPRELDEQQKAALAADITDVIIHHLNSKDSSISIALQQIQPESWQAIWDAEIAPQMEALIKKPGYSMNA

SEQ ID NO: 2 - DNA, 235 bp, Artificial Sequence
  pptA
atgccgcacatcgacattaaatgttttccgcgtgaactggacgaacaacaaaaagcagcacttgctgcagatattaccgacgttattattcatcatctgaacagtaaagacagttcgataagcattgctctacagcagattcaaccagaatcttggcaagctatctgggatgccgaaatcgcgccccaaatggaggctttgataaagaaacctggttatagcatgaatgcttaac

SEQ ID NO: 3 - protein, 77 aa, Unknown
  pptA
MPHIDIKCFPRELDEQQKAALAADITDVIIRHLNSKDSSISIALQQIQPESWQAIWDAEIAPQMEALIKKPGYSMNA

SEQ ID NO: 4 - DNA, 234 bp, Unknown
  pptA
atgccgcacatcgacattaaatgttttccgcgtgaactggacgaacaacaaaaagcagcacttgctgcagatattaccgacgttattattcgtcatctgaacagtaaagacagttcgataagcattgctctacagcagattcaaccagaatcttggcaagctatctgggatgccgaaatcgcgccccaaatggaggctttgataaagaaacctggttatagcatgaatgcttaa

SEQ ID NO: 5 - DNA, 40 bp, Artificial Sequence
  Forward Primer
ggaattcgagctcggtacccgagctcgaaatgacggtcag

SEQ ID NO: 6 - DNA, 21 bp, Artificial Sequence
  Reverse Primer
gttcagatgatgaataataac

SEQ ID NO: 7 - DNA, 21 bp, Artificial Sequence
  Forward Primer
gttattattcatcatctgaac

SEQ ID NO: 8 - DNA, 40 bp, Artificial Sequence
  Reverse Primer
gttatccctagcggatccccgcagcaactaactggacgtg

SEQ ID NO: 9 - DNA, 20 bp, Artificial Sequence
  Forward Primer
ttcggtccataatagcagaa

SEQ ID NO: 10 - DNA, 20 bp, Artificial Sequence
  Reverse Primer
ccagggagttgattgaacat